European Patent Specification EP 3 352 778 B1, published December 13, 2023. Title: METHODS, COMPOUNDS AND COMPOSITIONS FOR MODULATING BLOOD BRAIN BARRIER INTEGRITY AND RE-MYELINATION. Applicant: UNIVERSITY HEALTH NETWORK. Application N/A. The sequence listing filed with the application follows.

SEQUENCE LISTING (6 sequences)

SEQ ID NO: 1 - protein, 359 aa, Homo sapiens
CKILRCNAEYVSSTLSLRGGGSSGALRGGGGGGRGGGVGSGGLCRALRSYALCTRRTARTCRGDLAFHSAVHGIEDLMIQHNCSRQGPTAPPPPRGPALPGAGSGLPAPDPCDYEGRFSRLHGRPPGFLHCASFGDPHVRSFHHHFHTCRVQGAWPLLDNDFLFVQATSSPMALGANATATRKLTIIFKNMQECIDQKVYQAEVDNLPVAFEDGSINGGDRPGGSSLSIQTANPGNHVEIQAAYIGTTIIIRQTAGQLSFSIKVAEDVAMAFSAEQDLQLCVGGCPPSQRLSRSERNRRGAITIDTARRLCKEGLPVEDAYFHSCVFDVLISGDPNFTVAAQAALEDARAFLPDLEKLH

SEQ ID NO: 2 - DNA, 1077 bp, Homo sapiens
tgcaagatcctccgctgcaatgctgagtacgtatcgtccactctgagccttagaggtgggggttcatcaggagcacttcgaggaggaggaggaggaggccggggtggaggggtgggctctggcggcctctgtcgagccctccgctcctatgcgctctgcactcggcgcaccgcccgcacctgccgcggggacctcgccttccattcggcggtacatggcatcgaagacctgatgatccagcacaactgctcccgccagggccctacagcccctcccccgccccggggccccgcccttccaggcgcgggctccggcctccctgccccggacccttgtgactatgaaggccggttttcccggctgcatggtcgtcccccggggttcttgcattgcgcttccttcggggacccccatgtgcgcagcttccaccatcactttcacacatgccgtgtccaaggagcttggcctctactggataatgacttcctctttgtccaagccaccagctcccccatggcgttgggggccaacgctaccgccacccggaagctcaccatcatatttaagaacatgcaggaatgcattgatcagaaggtgtatcaggctgaggtggataatcttcctgtagcctttgaagatggttctatcaatggaggtgaccgacctgggggatccagtttgtcgattcaaactgctaaccctgggaaccatgtggagatccaagctgcctacattggcacaactataatcattcggcagacagctgggcagctctccttctccatcaaggtagcagaggatgtggccatggccttctcagctgaacaggacctgcagctctgtgttggggggtgccctccaagtcagcgactctctcgatcagagcgcaatcgtcggggagctataaccattgatactgccagacggctgtgcaaggaagggcttccagtggaagatgcttacttccattcctgtgtctttgatgttttaatttctggtgatcccaactttaccgtggcagctcaggcagcactggaggatgcccgagccttcctgccagacttagagaagctgcat

SEQ ID NO: 3 - protein, 357 aa, Mus musculus
CKILRCNAEYVSSTLSLRGGGSPDTPRGGGRGGLASGGLCRALRSYALCTRRTARTCRGDLAFHSAVHGIEDLMIQHNCSRQGPTAPPPARGPALPGAGPAPLTPDPCDYEARFSRLHGRAPGFLHCASFGDPHVRSFHNQFHTCRVQGAWPLLDNDFLFVQATSSPVSSGANATTIRKITIIFKNMQECIDQKVYQAEVDNLPAAFEDGSINGGDRPGGSSLSIQTANLGSHVEIRAAYIGTTIIIRQTAGQLSFSIRVAEDVARAFSAEQDLQLCVGGCPPSQRLSRSERNRRGAIAIDTARRLCKEGLPVEDAYFQSCVFDVSVSGDPNFTVAAQTALDDARIFLTDLENLHLF

SEQ ID NO: 4 - DNA, 1071 bp, Mus musculus
tgcaagatcctccgctgcaatgccgagtatgtctcgtccactctgagtcttcggggaggtggctcaccggacacgccgcgtggaggcggccgtggtgggctggcctcaggtggcttgtgtcgcgccctgcgctcctacgctctctgcacgcggcgcacggcccgcacctgccgcggggaccttgctttccactctgcggtgcatggcatagaggacctgatgatccagcacaactgctcacgccagggtcccacggccccgcccccggcccggggccccgccctgcccggggccgggccagcgcccctgaccccagatccctgtgactatgaggcccggttttccaggctgcacggtcgagccccgggcttcttgcattgcgcatcctttggagatccccatgtgcgcagtttccacaaccaatttcacacatgccgtgtccaaggagcttggcccttgctagataacgacttcctctttgtccaggccaccagctccccggtttcgtcgggagccaacgctaccaccatccggaagatcactatcatatttaaaaacatgcaggaatgcattgaccagaaagtctaccaggctgaggtggacaatcttcctgcagcctttgaagatggttctatcaatgggggcgaccgacctgggggctcgagtttgtccattcaaactgctaaccttgggagtcacgtggagattcgagctgcctacattggaacaactatcatcattcgacagacagctgggcagctctccttctccatcagggtagcagaggatgtggcgcgggccttctccgcagagcaggacctacagctgtgtgttgggggatgccctccgagccagcgactctctcgctcagagcgcaaccgccgtggggctatagccatagatactgccagaaggctgtgtaaggaagggcttccggttgaagatgcctacttccaatcctgcgtctttgatgtttcagtctccggtgaccccaactttactgtggcagctcagacagctctggacgatgcccgaatcttcttgacggatttagagaacttacatctcttt

SEQ ID NO: 5 - DNA, 47 bp, Artificial Sequence
  Forward Primer
cttggtacccatcatcatcatcatcatcagtgcaagatcctccgctg

SEQ ID NO: 6 - DNA, 41 bp, Artificial Sequence
  Reverse Primer
gcgtctagacactcgagcgtcgagctgcccagctgtctgtc